European Patent Application EP 4 772 539 A1, published July 8, 2026. Title: CTLA4/TIGIT结合蛋白及其医药用途. Applicant: 江苏恒瑞医药股份有限公司. Application WO. The sequence listing filed with the application follows.

SEQUENCE LISTING (52 sequences)

SEQ ID NO: 1 - protein, 5 aa, synthetic construct
  source 1..5: note = CDR
SYTMH

SEQ ID NO: 2 - protein, 17 aa, synthetic construct
  source 1..17: note = CDR
FISYDGNNKYYADSVKG

SEQ ID NO: 3 - protein, 9 aa, synthetic construct
  source 1..9: note = CDR
TGWLGPFDY

SEQ ID NO: 4 - protein, 12 aa, synthetic construct
  source 1..12: note = CDR
RASQSVGSSYLA

SEQ ID NO: 5 - protein, 7 aa, synthetic construct
  source 1..7: note = CDR
GAFSRAT

SEQ ID NO: 6 - protein, 9 aa, synthetic construct
  source 1..9: note = CDR
QQYGSSPWT

SEQ ID NO: 7 - protein, 5 aa, synthetic construct
  source 1..5: note = CDR
NYWMH

SEQ ID NO: 8 - protein, 17 aa, synthetic construct
  source 1..17: note = CDR
RIDPDSTGSKYNEKFKT

SEQ ID NO: 9 - protein, 10 aa, synthetic construct
  source 1..10: note = CDR
EGAYGYYFDY

SEQ ID NO: 10 - protein, 11 aa, synthetic construct
  source 1..11: note = CDR
RASENIYSYLA

SEQ ID NO: 11 - protein, 7 aa, synthetic construct
  source 1..7: note = CDR
NARTLAE

SEQ ID NO: 12 - protein, 9 aa, synthetic construct
  source 1..9: note = CDR
QYHSGSPLP

SEQ ID NO: 13 - protein, 118 aa, synthetic construct
  source 1..118: note = As-3 VH1
QVQLVESGGGVVQPGRSLRLSCAASGFTFSSYTMHWVRQAPGKGLEWVTFISYDGNNKYYADSVKGRFTISRDNSKNTLYLQMNSLRAEDTAIYYCARTGWLGPFDYWGQGTLVTVSS

SEQ ID NO: 14 - protein, 108 aa, synthetic construct
  source 1..108: note = As-3 VL1
EIVLTQSPGTLSLSPGERATLSCRASQSVGSSYLAWYQQKPGQAPRLLIYGAFSRATGIPDRFSGSGSGTDFTLTISRLEPEDFAVYYCQQYGSSPWTFGQGTKVEIK

SEQ ID NO: 15 - protein, 119 aa, synthetic construct
  source 1..119: note = As-3 VH2
EVQLVQSGAEVKKPGASVKVSCKASGYTFTNYWMHWVRQAPGQGLEWMGRIDPDSTGSKYNEKFKTRVTMTRDTSTSTVYMELSSLRSEDTAVYYCAREGAYGYYFDYWGQGTLVTVSS

SEQ ID NO: 16 - protein, 107 aa, synthetic construct
  source 1..107: note = As-3 VL2
DIQMTQSPSSLSASVGDRVTITCRASENIYSYLAWYQQKPGKSPKLLIYNARTLAEGVPSRFSGSGSGTDFTLTISSLQPEDFATYYCQYHSGSPLPFGGGTKVEIK

SEQ ID NO: 17 - protein, 97 aa, synthetic construct
  source 1..97: note = Obscurin-O
SGAPRFLTRPKASVVSVGKDATLSCQIVGNPFPQVSWEKDKQPVTAGVRFRLAQDGDLYRLKILDLQLSDSGQYVCRARNAHGEAFACLGLQVDAEA

SEQ ID NO: 18 - protein, 98 aa, synthetic construct
  source 1..98: note = Titin-T
GIPPKIECLPIDISIDEGKVLTVASAFTGEPTPEVTWSTGGRKIHSQEQGRFHIENTDDSTTLTIKDVQKQDGGLYTLTLRNEFGSDSATVNIHIRSI

SEQ ID NO: 19 - protein, 103 aa, synthetic construct
  source 1..103: note = CH1
ASTKGPSVFPLAPSSKSTSGGTAALGCLVKDYFPEPVTVSWNSGALTSGVHTFPAVLQSSGLYSLSSVVTVPSSSLGTQTYICNVNHKPSNTKVDKKVEPKSC

SEQ ID NO: 20 - protein, 107 aa, synthetic construct [sequence omitted]

SEQ ID NO: 21 - protein, 447 aa, synthetic construct
  source 1..447: note = As-3 H1
QVQLVESGGGVVQPGRSLRLSCAASGFTFSSYTMHWVRQAPGKGLEWVTFISYDGNNKYYADSVKGRFTISRDNSKNTLYLQMNSLRAEDTAIYYCARTGWLGPFDYWGQGTLVTVSSGGGGSSGAPRFLTRPKASVVSVGKDATLSCQIVGNPFPQVSWEKDKQPVTAGVRFRLAQDGDLYRLKILDLQLSDSGQYVCRARNAHGEAFACLGLQVDAEADKTHTCPPCPAPELLGGPDVFLFPPKPKDTLMISRTPEVTCVVVDVSHEDPEVKFNWYVDGVEVHNAKTKPREEQYNSTYRVVSVLTVLHQDWLNGKEYKCKVSNKALPLPEEKTISKAKGQPREPQVYTLPPCREEMTKNQVSLWCLVKGFYPSDIAVEWESNGQPENNYKTTPPVLDSDGSFFLYSKLTVDKSRWQQGNVFSCSVMHEALHNHYTQKSLSLSPGK

SEQ ID NO: 22 - protein, 211 aa, synthetic construct
  source 1..211: note = As-3 L1
EIVLTQSPGTLSLSPGERATLSCRASQSVGSSYLAWYQQKPGQAPRLLIYGAFSRATGIPDRFSGSGSGTDFTLTISRLEPEDFAVYYCQQYGSSPWTFGQGTKVEIKGGGGSGIPPKIECLPIDISIDEGKVLTVASAFTGEPTPEVTWSTGGRKIHSQEQGRFHIENTDDSTTLTIKDVQKQDGGLYTLTLRNEFGSDSATVNIHIRSI

SEQ ID NO: 23 - protein, 449 aa, synthetic construct
  source 1..449: note = As-3 H2
EVQLVQSGAEVKKPGASVKVSCKASGYTFTNYWMHWVRQAPGQGLEWMGRIDPDSTGSKYNEKFKTRVTMTRDTSTSTVYMELSSLRSEDTAVYYCAREGAYGYYFDYWGQGTLVTVSSASTKGPSVFPLAPSSKSTSGGTAALGCLVKDYFPEPVTVSWNSGALTSGVHTFPAVLQSSGLYSLSSVVTVPSSSLGTQTYICNVNHKPSNTKVDKKVEPKSCDKTHTCPPCPAPELLGGPDVFLFPPKPKDTLMISRTPEVTCVVVDVSHEDPEVKFNWYVDGVEVHNAKTKPREEQYNSTYRVVSVLTVLHQDWLNGKEYKCKVSNKALPLPEEKTISKAKGQPREPQVCTLPPSREEMTKNQVSLSCAVKGFYPSDIAVEWESNGQPENNYKTTPPVLDSDGSFFLVSKLTVDKSRWQQGNVFSCSVMHEALHNHYTQKSLSLSPGK

SEQ ID NO: 24 - protein, 214 aa, synthetic construct
  source 1..214: note = As-3 L2
DIQMTQSPSSLSASVGDRVTITCRASENIYSYLAWYQQKPGKSPKLLIYNARTLAEGVPSRFSGSGSGTDFTLTISSLQPEDFATYYCQYHSGSPLPFGGGTKVEIKRTVAAPSVFIFPPSDEQLKSGTASVVCLLNNFYPREAKVQWKVDNALQSGNSQESVTEQDSKDSTYSLSSTLTLSKADYEKHKVYACEVTHQGLSSPVTKSFNRGEC

SEQ ID NO: 25 - protein, 227 aa, synthetic construct
  source 1..227: note = IgG1 Fc1
DKTHTCPPCPAPELLGGPDVFLFPPKPKDTLMISRTPEVTCVVVDVSHEDPEVKFNWYVDGVEVHNAKTKPREEQYNSTYRVVSVLTVLHQDWLNGKEYKCKVSNKALPLPEEKTISKAKGQPREPQVYTLPPCREEMTKNQVSLWCLVKGFYPSDIAVEWESNGQPENNYKTTPPVLDSDGSFFLYSKLTVDKSRWQQGNVFSCSVMHEALHNHYTQKSLSLSPGK

SEQ ID NO: 26 - protein, 227 aa, synthetic construct
  source 1..227: note = IgG1 Fc2
DKTHTCPPCPAPELLGGPDVFLFPPKPKDTLMISRTPEVTCVVVDVSHEDPEVKFNWYVDGVEVHNAKTKPREEQYNSTYRVVSVLTVLHQDWLNGKEYKCKVSNKALPLPEEKTISKAKGQPREPQVCTLPPSREEMTKNQVSLSCAVKGFYPSDIAVEWESNGQPENNYKTTPPVLDSDGSFFLVSKLTVDKSRWQQGNVFSCSVMHEALHNHYTQKSLSLSPGK

SEQ ID NO: 27 - protein, 5 aa, synthetic construct
  source 1..5: note = CDR
SYGMH

SEQ ID NO: 28 - protein, 17 aa, synthetic construct
  source 1..17: note = CDR
VIWYDGSNKYYADSVKG

SEQ ID NO: 29 - protein, 16 aa, synthetic construct
  source 1..16: note = CDR
DPRGATLYYYYYGMDV

SEQ ID NO: 30 - protein, 11 aa, synthetic construct
  source 1..11: note = CDR
RASQSINSYLD

SEQ ID NO: 31 - protein, 7 aa, synthetic construct
  source 1..7: note = CDR
AASSLQS

SEQ ID NO: 32 - protein, 9 aa, synthetic construct
  source 1..9: note = CDR
QQYYSTPFT

SEQ ID NO: 33 - protein, 692 aa, synthetic construct
  source 1..692: note = S-15 H1
EVQLVQSGAEVKKPGASVKVSCKASGYTFTNYWMHWVRQAPGQGLEWMGRIDPDSTGSKYNEKFKTRVTMTRDTSTSTVYMELSSLRSEDTAVYYCAREGAYGYYFDYWGQGTLVTVSSASTKGPSVFPLAPSSKSTSGGTAALGCLVKDYFPEPVTVSWNSGALTSGVHTFPAVLQSSGLYSLSSVVTVPSSSLGTQTYICNVNHKPSNTKVDKKVEPKSCDGGGGSGGGGSGGGGSQVQLVESGGGVVQPGRSLRLSCAASGFTFSSYGMHWVRQAPGKGLEWVAVIWYDGSNKYYADSVKGRFTISRDNSKNTLYLQMNSLRAEDTAVYYCARDPRGATLYYYYYGMDVWGQGTTVTVSSGGGGSSGAPRFLTRPKASVVSVGKDATLSCQIVGNPFPQVSWEKDKQPVTAGVRFRLAQDGDLYRLKILDLQLSDSGQYVCRARNAHGEAFACLGLQVDAEADKTHTCPPCPAPELLGGPDVFLFPPKPKDTLMISRTPEVTCVVVDVSHEDPEVKFNWYVDGVEVHNAKTKPREEQYNSTYRVVSVLTVLHQDWLNGKEYKCKVSNKALPLPEEKTISKAKGQPREPQVYTLPPSREEMTKNQVSLTCLVKGFYPSDIAVEWESNGQPENNYKTTPPVLDSDGSFFLYSKLTVDKSRWQQGNVFSCSVMHEALHNHYTQKSLSLSPGK

SEQ ID NO: 34 - protein, 214 aa, synthetic construct; identical to SEQ ID NO: 24
  source 1..214: note = S-15 L1

SEQ ID NO: 35 - protein, 210 aa, synthetic construct
  source 1..210: note = S-15 L2
DIQMTQSPSSLSASVGDRVTITCRASQSINSYLDWYQQKPGKAPKLLIYAASSLQSGVPSRFSGSGSGTDFTLTISSLQPEDFATYYCQQYYSTPFTFGPGTKVEIKGGGGSGIPPKIECLPIDISIDEGKVLTVASAFTGEPTPEVTWSTGGRKIHSQEQGRFHIENTDDSTTLTIKDVQKQDGGLYTLTLRNEFGSDSATVNIHIRSI

SEQ ID NO: 36 - protein, 448 aa, synthetic construct
  source 1..448: note = Ipilimumab HC
QVQLVESGGGVVQPGRSLRLSCAASGFTFSSYTMHWVRQAPGKGLEWVTFISYDGNNKYYADSVKGRFTISRDNSKNTLYLQMNSLRAEDTAIYYCARTGWLGPFDYWGQGTLVTVSSASTKGPSVFPLAPSSKSTSGGTAALGCLVKDYFPEPVTVSWNSGALTSGVHTFPAVLQSSGLYSLSSVVTVPSSSLGTQTYICNVNHKPSNTKVDKKVEPKSCDKTHTCPPCPAPELLGGPSVFLFPPKPKDTLMISRTPEVTCVVVDVSHEDPEVKFNWYVDGVEVHNAKTKPREEQYNSTYRVVSVLTVLHQDWLNGKEYKCKVSNKALPAPIEKTISKAKGQPREPQVYTLPPSREEMTKNQVSLTCLVKGFYPSDIAVEWESNGQPENNYKTTPPVLDSDGSFFLYSKLTVDKSRWQQGNVFSCSVMHEALHNHYTQKSLSLSPGK

SEQ ID NO: 37 - protein, 215 aa, synthetic construct
  source 1..215: note = Ipilimumab LC
EIVLTQSPGTLSLSPGERATLSCRASQSVGSSYLAWYQQKPGQAPRLLIYGAFSRATGIPDRFSGSGSGTDFTLTISRLEPEDFAVYYCQQYGSSPWTFGQGTKVEIKRTVAAPSVFIFPPSDEQLKSGTASVVCLLNNFYPREAKVQWKVDNALQSGNSQESVTEQDSKDSTYSLSSTLTLSKADYEKHKVYACEVTHQGLSSPVTKSFNRGEC

SEQ ID NO: 38 - protein, 449 aa, synthetic construct
  source 1..449: note = S2 HC
EVQLVQSGAEVKKPGASVKVSCKASGYTFTNYWMHWVRQAPGQGLEWMGRIDPDSTGSKYNEKFKTRVTMTRDTSTSTVYMELSSLRSEDTAVYYCAREGAYGYYFDYWGQGTLVTVSSASTKGPSVFPLAPSSKSTSGGTAALGCLVKDYFPEPVTVSWNSGALTSGVHTFPAVLQSSGLYSLSSVVTVPSSSLGTQTYICNVNHKPSNTKVDKKVEPKSCDKTHTCPPCPAPELLGGPSVFLFPPKPKDTLMISRTPEVTCVVVDVSHEDPEVKFNWYVDGVEVHNAKTKPREEQYNSTYRVVSVLTVLHQDWLNGKEYKCKVSNKALPAPIEKTISKAKGQPREPQVYTLPPSREEMTKNQVSLTCLVKGFYPSDIAVEWESNGQPENNYKTTPPVLDSDGSFFLYSKLTVDKSRWQQGNVFSCSVMHEALHNHYTQKSLSLSPGK

SEQ ID NO: 39 - protein, 214 aa, synthetic construct; identical to SEQ ID NO: 24
  source 1..214: note = S2 LC

SEQ ID NO: 40 - protein, 455 aa, synthetic construct
  source 1..455: note = Tre HC
QVQLVESGGGVVQPGRSLRLSCAASGFTFSSYGMHWVRQAPGKGLEWVAVIWYDGSNKYYADSVKGRFTISRDNSKNTLYLQMNSLRAEDTAVYYCARDPRGATLYYYYYGMDVWGQGTTVTVSSASTKGPSVFPLAPSSKSTSGGTAALGCLVKDYFPEPVTVSWNSGALTSGVHTFPAVLQSSGLYSLSSVVTVPSSSLGTQTYICNVNHKPSNTKVDKKVEPKSCDKTHTCPPCPAPELLGGPSVFLFPPKPKDTLMISRTPEVTCVVVDVSHEDPEVKFNWYVDGVEVHNAKTKPREEQYNSTYRVVSVLTVLHQDWLNGKEYKCKVSNKALPAPIEKTISKAKGQPREPQVYTLPPSREEMTKNQVSLTCLVKGFYPSDIAVEWESNGQPENNYKTTPPVLDSDGSFFLYSKLTVDKSRWQQGNVFSCSVMHEALHNHYTQKSLSLSPGK

SEQ ID NO: 41 - protein, 214 aa, synthetic construct
  source 1..214: note = Tre LC
DIQMTQSPSSLSASVGDRVTITCRASQSINSYLDWYQQKPGKAPKLLIYAASSLQSGVPSRFSGSGSGTDFTLTISSLQPEDFATYYCQQYYSTPFTFGPGTKVEIKRTVAAPSVFIFPPSDEQLKSGTASVVCLLNNFYPREAKVQWKVDNALQSGNSQESVTEQDSKDSTYSLSSTLTLSKADYEKHKVYACEVTHQGLSSPVTKSFNRGEC

SEQ ID NO: 42 - protein, 456 aa, synthetic construct
  source 1..456: note = RG6058 HC
EVQLQQSGPGLVKPSQTLSLTCAISGDSVSSNSAAWNWIRQSPSRGLEWLGKTYYRFKWYSDYAVSVKGRITINPDTSKNQFSLQLNSVTPEDTAVFYCTRESTTYDLLAGPFDYWGQGTLVTVSSASTKGPSVFPLAPSSKSTSGGTAALGCLVKDYFPEPVTVSWNSGALTSGVHTFPAVLQSSGLYSLSSVVTVPSSSLGTQTYICNVNHKPSNTKVDKKVEPKSCDKTHTCPPCPAPELLGGPSVFLFPPKPKDTLMISRTPEVTCVVVDVSHEDPEVKFNWYVDGVEVHNAKTKPREEQYNSTYRVVSVLTVLHQDWLNGKEYKCKVSNKALPAPIEKTISKAKGQPREPQVYTLPPSREEMTKNQVSLTCLVKGFYPSDIAVEWESNGQPENNYKTTPPVLDSDGSFFLYSKLTVDKSRWQQGNVFSCSVMHEALHNHYTQKSLSLSPGK

SEQ ID NO: 43 - protein, 220 aa, synthetic construct
  source 1..220: note = RG6058 LC
DIVMTQSPDSLAVSLGERATINCKSSQTVLYSSNNKKYLAWYQQKPGQPPNLLIYWASTRESGVPDRFSGSGSGTDFTLTISSLQAEDVAVYYCQQYYSTPFTFGPGTKVEIKRTVAAPSVFIFPPSDEQLKSGTASVVCLLNNFYPREAKVQWKVDNALQSGNSQESVTEQDSKDSTYSLSSTLTLSKADYEKHKVYACEVTHQGLSSPVTKSFNRGEC

SEQ ID NO: 44 - protein, 5 aa, synthetic construct
  source 1..5: note = linker
GGNGT

SEQ ID NO: 45 - protein, 5 aa, synthetic construct
  source 1..5: note = linker
YGNGT

SEQ ID NO: 46 - protein, 5 aa, synthetic construct
  source 1..5: note = linker
EPKSS

SEQ ID NO: 47 - protein, 5 aa, synthetic construct
  source 1..5: note = linker
GGGGS

SEQ ID NO: 48 - protein, 10 aa, synthetic construct
  source 1..10: note = linker
GGGGSGGGGS

SEQ ID NO: 49 - protein, 15 aa, synthetic construct
  source 1..15: note = linker
GGGGSGGGGSGGGGS

SEQ ID NO: 50 - protein, 20 aa, synthetic construct
  source 1..20: note = linker
GGGGSGGGGSGGGGSGGGGS

SEQ ID NO: 51 - protein, 25 aa, synthetic construct
  source 1..25: note = linker
GGGGSGGGGSGGGGSGGGGSGGGGS

SEQ ID NO: 52 - protein, 4 aa, synthetic construct
  source 1..4: note = linker
ASGS